European Patent Application EP 4 678 648 A1, published January 14, 2026. Title: 근접 효과 기반 위치 선택적 항체 표지를 이용한 항체-약물 접합체의 합성 방법. Applicant: 서강대학교산학협력단. Application KR. The sequence listing filed with the application follows.

SEQUENCE LISTING (8 sequences)

SEQ ID NO: 1 - protein, 67 aa, synthetic construct
MVDNKFNKEQQNAFYEILHLPNLNEEQRNAFIQSLKDDPSQSANLLAEAKKLNDAQAPKGSHHHHHH

SEQ ID NO: 2 - protein, 67 aa, synthetic construct
MVDNKFNMQQQRRFYEALHDPNLNEEQRNAKIKSIRDDPSQSANLLAEAKKLNDAQAPKGSHHHHHH

SEQ ID NO: 3 - protein, 67 aa, synthetic construct
  VARIANT 8: note = X is AzK
MVDNKFNXQQQRRFYEALHDPNLNEEQRNAKIKSIRDDPSQSANLLAEAKKLNDAQAPKGSHHHHHH

SEQ ID NO: 4 - protein, 11 aa, synthetic construct
KGSVDNKFNKE

SEQ ID NO: 5 - protein, 228 aa, synthetic construct
ASDKTHTCPPCPAPELLGGPSVFLFPPKPKDTLMISRTPEVTCVVVDVSHEDPEVKFNWYVDGVEVHNAKTKPREEQYNSTYRVVSVLTVLHQDWLNGKEYKCKVSNKALPAPIEKTISKAKGQPREPQVYTLPPSREEMTKNQVSLTCLVKGFYPSDIAVEWESNGQPENNYKTTPPVLDSDGSFFLYSKLTVDKSRWQQGNVFSCSVMHEALHNHYTQKSLSLSPG

SEQ ID NO: 6 - protein, 37 aa, synthetic construct
ASDKTHTCPPCPAPELLGGPSVFLFPPKPKDTLMISR

SEQ ID NO: 7 - protein, 450 aa, synthetic construct
EVQLVESGGGLVQPGGSLRLSCAASGFNIKDTYIHWVRQAPGKGLEWVARIYPTNGYTRYADSVKGRFTISADTSKNTAYLQMNSLRAEDTAVYYCSRWGGDGFYAMDYWGQGTLVTVSSASTKGPSVFPLAPSSKSTSGGTAALGCLVKDYFPEPVTVSWNSGALTSGVHTFPAVLQSSGLYSLSSVVTVPSSSLGTQTYICNVNHKPSNTKVDKKVEPKSCDKTHTCPPCPAPELLGGPSVFLFPPKPKDTLMISRTPEVTCVVVDVSHEDPEVKFNWYVDGVEVHNAKTKPREEQYNSTYRVVSVLTVLHQDWLNGKEYKCKVSNKALPAPIEKTISKAKGQPREPQVYTLPPSREEMTKNQVSLTCLVKGFYPSDIAVEWESNGQPENNYKTTPPVLDSDGSFFLYSKLTVDKSRWQQGNVFSCSVMHEALHNHYTQKSLSLSPGK

SEQ ID NO: 8 - protein, 19 aa, synthetic construct
GPSVFLFPPKPKDTLMISR